European Patent Application EP 4 365 194 A2, published May 8, 2024. Title: CD79A CHIMERIC ANTIGEN RECEPTORS. Applicant: 2Seventy bio, Inc. Application WO PCT/US2019/037270, filed June 14, 2019. The sequence listing filed with the application follows.

SEQUENCE LISTING (79 sequences)

SEQ ID NO: 1 - protein, 16 aa, synthetic construct
  REGION 1..16: note = Made in Lab - Light chain CDR1
RSSQSIVHSNGNTYLE

SEQ ID NO: 2 - protein, 7 aa, synthetic construct
  REGION 1..7: note = Made in Lab - Light chain CDR2
KVSNRFS

SEQ ID NO: 3 - protein, 9 aa, synthetic construct
  REGION 1..9: note = Made in Lab - Light Chain CDR3
FQGSHVPFT

SEQ ID NO: 4 - protein, 10 aa, synthetic construct
  REGION 1..10: note = Made in Lab - Heavy chain CDR1
GYTFSTSWMN

SEQ ID NO: 5 - protein, 17 aa, synthetic construct
  REGION 1..17: note = Made in Lab - Heavy chain CDR2
RIYPGDGDTNYNGKFKG

SEQ ID NO: 6 - protein, 11 aa, synthetic construct
  REGION 1..11: note = Made in Lab - Heavy chain CDR6
FYYGNTFAMDY

SEQ ID NO: 7 - protein, 112 aa, synthetic construct
  REGION 1..112: note = Made in Lab - Varialble light chain
DVLMTQIPLSLPVSLGDQASISCRSSQSIVHSNGNTYLEWYLQKPGQSPKLLIYKVSNRFSGVPDRFSGSGSGTDFTLKISRVEAEDLGVYYCFQGSHVPFTFGSGTKLEIK

SEQ ID NO: 8 - protein, 120 aa, synthetic construct
  REGION 1..120: note = Made in Lab - Variable heavy chain
QVQLQQSGPELVKPGASVKISCKASGYTFSTSWMNWVKQRPGQGLEWIGRIYPGDGDTNYNGKFKGKATLTADKSSNTAYMQLSSLTSVDSAVYFCERFYYGNTFAMDYWGQGTSVTVSS

SEQ ID NO: 9 - protein, 16 aa, synthetic construct
  REGION 1..16: note = Made in Lab - Light chain CDR1
RSSQSLVHSNGNTYLH

SEQ ID NO: 10 - protein, 7 aa, synthetic construct
  REGION 1..7: note = Made in Lab - Light chain CDR2
KVSNRFS

SEQ ID NO: 11 - protein, 10 aa, synthetic construct
  REGION 1..10: note = Made in Lab - Light Chain CDR3
SQSTHVPPYT

SEQ ID NO: 12 - protein, 10 aa, synthetic construct
  REGION 1..10: note = Made in Lab - Heavy chain CDR1
GYAFSFSWMN

SEQ ID NO: 13 - protein, 17 aa, synthetic construct
  REGION 1..17: note = Made in Lab - Heavy chain CDR2
RIYPGNGDTNYNGKFKG

SEQ ID NO: 14 - protein, 12 aa, synthetic construct
  REGION 1..12: note = Made in Lab - Heavy chain CDR6
WVYSGNNYAVDY

SEQ ID NO: 15 - protein, 113 aa, synthetic construct
  REGION 1..113: note = Made in Lab - Varialble light chain
DVVMTQTPLSLPVSLGDQASISCRSSQSLVHSNGNTYLHWYLQKPGQSPKLLIYKVSNRFSGVPDRFSGSGSGTDFTLKISRVEAEDLGVYFCSQSTHVPPYTFGGGTKLEIK

SEQ ID NO: 16 - protein, 121 aa, synthetic construct
  REGION 1..121: note = Made in Lab - Variable heavy chain
QVQLQQSGPELVKPGASVKISCKTSGYAFSFSWMNWVKWGPGQGLEWIGRIYPGNGDTNYNGKFKGKATLTADKSSNTAYMQLSSLTSVDSAVYFCARWVYSGNNYAVDYWGQGTSVTVSS

SEQ ID NO: 17 - protein, 14 aa, synthetic construct
  REGION 1..14: note = Made in Lab - Light chain CDR1
TGTSSDFGSYNLVS

SEQ ID NO: 18 - protein, 7 aa, synthetic construct
  REGION 1..7: note = Made in Lab - Light chain CDR2
EGSKRPS

SEQ ID NO: 19 - protein, 10 aa, synthetic construct
  REGION 1..10: note = Made in Lab - Light Chain CDR3
CSYAGGSTWV

SEQ ID NO: 20 - protein, 10 aa, synthetic construct
  REGION 1..10: note = Made in Lab - Heavy chain CDR1
GLTFTSYAMN

SEQ ID NO: 21 - protein, 17 aa, synthetic construct
  REGION 1..17: note = Made in Lab - Heavy chain CDR2
GISGSGGGTYYADSVKG

SEQ ID NO: 22 - protein, 7 aa, synthetic construct
  REGION 1..7: note = Made in Lab - Heavy chain CDR6
LGGWSDY

SEQ ID NO: 23 - protein, 110 aa, synthetic construct
  REGION 1..110: note = Made in Lab - Varialble light chain
QSALTQPASVSGSPGQSITISCTGTSSDFGSYNLVSWYQQHPGKAPKLMIYEGSKRPSGVSNRFSGSKSGNTASLTISGLQAEDEADYYCCSYAGGSTWVFGGGTKLTVL

SEQ ID NO: 24 - protein, 116 aa, synthetic construct
  REGION 1..116: note = Made in Lab - Variable heavy chain
EVQLLESGGGLVQPGGSLRLSCAASGLTFTSYAMNWVRQAPGKGLEWVSGISGSGGGTYYADSVKGRFTISRDNSKNTLYLQMNSLRAEDTAVYYCAKLGGWSDYWGQGTLVTVSS

SEQ ID NO: 25 - protein, 492 aa, synthetic construct
  REGION 1..492: note = Made in Lab - anti-CD79A-01_HL CAR construct
MALPVTALLLPLALLLHAARPQVQLQQSGPELVKPGASVKISCKASGYTFSTSWMNWVKQRPGQGLEWIGRIYPGDGDTNYNGKFKGKATLTADKSSNTAYMQLSSLTSVDSAVYFCERFYYGNTFAMDYWGQGTSVTVSSGGGGSGGGGSGGGGSDVLMTQIPLSLPVSLGDQASISCRSSQSIVHSNGNTYLEWYLQKPGQSPKLLIYKVSNRFSGVPDRFSGSGSGTDFTLKISRVEAEDLGVYYCFQGSHVPFTFGSGTKLEIKRTTTPAPRPPTPAPTIASQPLSLRPEACRPAAGGAVHTRGLDFACDIYIWAPLAGTCGVLLLSLVITLYCKRGRKKLLYIFKQPFMRPVQTTQEEDGCSCRFPEEEEGGCELRVKFSRSADAPAYQQGQNQLYNELNLGRREEYDVLDKRRGRDPEMGGKPRRKNPQEGLYNELQKDKMAEAYSEIGMKGERRRGKGHDGLYQGLSTATKDTYDALHMQALPPR

SEQ ID NO: 26 - protein, 492 aa, synthetic construct
  REGION 1..492: note = Made in Lab - anti-CD79A-01_LH CAR construct
MALPVTALLLPLALLLHAARPDVLMTQIPLSLPVSLGDQASISCRSSQSIVHSNGNTYLEWYLQKPGQSPKLLIYKVSNRFSGVPDRFSGSGSGTDFTLKISRVEAEDLGVYYCFQGSHVPFTFGSGTKLEIKRGGGGSGGGGSGGGGSQVQLQQSGPELVKPGASVKISCKASGYTFSTSWMNWVKQRPGQGLEWIGRIYPGDGDTNYNGKFKGKATLTADKSSNTAYMQLSSLTSVDSAVYFCERFYYGNTFAMDYWGQGTSVTVSSTTTPAPRPPTPAPTIASQPLSLRPEACRPAAGGAVHTRGLDFACDIYIWAPLAGTCGVLLLSLVITLYCKRGRKKLLYIFKQPFMRPVQTTQEEDGCSCRFPEEEEGGCELRVKFSRSADAPAYQQGQNQLYNELNLGRREEYDVLDKRRGRDPEMGGKPRRKNPQEGLYNELQKDKMAEAYSEIGMKGERRRGKGHDGLYQGLSTATKDTYDALHMQALPPR

SEQ ID NO: 27 - protein, 493 aa, synthetic construct
  REGION 1..493: note = Made in Lab - anti-CD79A-10_HL CAR construct
MALPVTALLLPLALLLHAARPQVQLQQSGPELVKPGASVKISCKTSGYAFSFSWMNWVKWGPGQGLEWIGRIYPGNGDTNYNGKFKGKATLTADKSSNTAYMQLSSLTSVDSAVYFCARWVYSGNNYAVDYWGQGTSVTVSSGGGGSGGGGSGGGGSDVVMTQTPLSLPVSLGDQASISCRSSQSLVHSNGNTYLHWYLQKPGQSPKLLIYKVSNRFSGVPDRFSGSGSGTDFTLKISRVEAEDLGVYFCSQSTHVPPYTFGGGTKLEIKTTTPAPRPPTPAPTIASQPLSLRPEACRPAAGGAVHTRGLDFACDIYIWAPLAGTCGVLLLSLVITLYCKRGRKKLLYIFKQPFMRPVQTTQEEDGCSCRFPEEEEGGCELRVKFSRSADAPAYQQGQNQLYNELNLGRREEYDVLDKRRGRDPEMGGKPRRKNPQEGLYNELQKDKMAEAYSEIGMKGERRRGKGHDGLYQGLSTATKDTYDALHMQALPPR

SEQ ID NO: 28 - protein, 493 aa, synthetic construct
  REGION 1..493: note = Made in Lab - anti-CD79A-10_LH CAR construct
MALPVTALLLPLALLLHAARPDVVMTQTPLSLPVSLGDQASISCRSSQSLVHSNGNTYLHWYLQKPGQSPKLLIYKVSNRFSGVPDRFSGSGSGTDFTLKISRVEAEDLGVYFCSQSTHVPPYTFGGGTKLEIKGGGGSGGGGSGGGGSQVQLQQSGPELVKPGASVKISCKTSGYAFSFSWMNWVKWGPGQGLEWIGRIYPGNGDTNYNGKFKGKATLTADKSSNTAYMQLSSLTSVDSAVYFCARWVYSGNNYAVDYWGQGTSVTVSSTTTPAPRPPTPAPTIASQPLSLRPEACRPAAGGAVHTRGLDFACDIYIWAPLAGTCGVLLLSLVITLYCKRGRKKLLYIFKQPFMRPVQTTQEEDGCSCRFPEEEEGGCELRVKFSRSADAPAYQQGQNQLYNELNLGRREEYDVLDKRRGRDPEMGGKPRRKNPQEGLYNELQKDKMAEAYSEIGMKGERRRGKGHDGLYQGLSTATKDTYDALHMQALPPR

SEQ ID NO: 29 - protein, 485 aa, synthetic construct
  REGION 1..485: note = Made in Lab - anti-CD79A-02_HL CAR construct
MALPVTALLLPLALLLHAARPEVQLLESGGGLVQPGGSLRLSCAASGLTFTSYAMNWVRQAPGKGLEWVSGISGSGGGTYYADSVKGRFTISRDNSKNTLYLQMNSLRAEDTAVYYCAKLGGWSDYWGQGTLVTVSSGGGGSGGGGSGGGGSQSALTQPASVSGSPGQSITISCTGTSSDFGSYNLVSWYQQHPGKAPKLMIYEGSKRPSGVSNRFSGSKSGNTASLTISGLQAEDEADYYCCSYAGGSTWVFGGGTKLTVLTTTPAPRPPTPAPTIASQPLSLRPEACRPAAGGAVHTRGLDFACDIYIWAPLAGTCGVLLLSLVITLYCKRGRKKLLYIFKQPFMRPVQTTQEEDGCSCRFPEEEEGGCELRVKFSRSADAPAYQQGQNQLYNELNLGRREEYDVLDKRRGRDPEMGGKPRRKNPQEGLYNELQKDKMAEAYSEIGMKGERRRGKGHDGLYQGLSTATKDTYDALHMQALPPR

SEQ ID NO: 30 - protein, 485 aa, synthetic construct
  REGION 1..485: note = Made in Lab - anti-CD79A-02_LH CAR construct
MALPVTALLLPLALLLHAARPQSALTQPASVSGSPGQSITISCTGTSSDFGSYNLVSWYQQHPGKAPKLMIYEGSKRPSGVSNRFSGSKSGNTASLTISGLQAEDEADYYCCSYAGGSTWVFGGGTKLTVLGGGGSGGGGSGGGGSEVQLLESGGGLVQPGGSLRLSCAASGLTFTSYAMNWVRQAPGKGLEWVSGISGSGGGTYYADSVKGRFTISRDNSKNTLYLQMNSLRAEDTAVYYCAKLGGWSDYWGQGTLVTVSSTTTPAPRPPTPAPTIASQPLSLRPEACRPAAGGAVHTRGLDFACDIYIWAPLAGTCGVLLLSLVITLYCKRGRKKLLYIFKQPFMRPVQTTQEEDGCSCRFPEEEEGGCELRVKFSRSADAPAYQQGQNQLYNELNLGRREEYDVLDKRRGRDPEMGGKPRRKNPQEGLYNELQKDKMAEAYSEIGMKGERRRGKGHDGLYQGLSTATKDTYDALHMQALPPR

SEQ ID NO: 31 - DNA, 1479 bp, synthetic construct
  misc_feature 1..1479: note = Made in Lab - anti-CD79A-01_HL CAR polynucleotide construct
  source 1..1479: mol_type = other DNA
atggcacttccagtgactgcattgttgttgcccctggccctgctgcttcacgccgcaaggccccaggtccagcttcagcagtccggaccagagttggtgaaacctggggcatcagtcaagattagctgcaaggcatcagggtacaccttcagcactagttggatgaattgggtgaagcagcggcctggccaggggttggagtggatcggacgcatctacccaggggatggcgatacaaactacaacggaaagtttaaaggtaaggctactttgaccgctgacaaatcatcaaacacggcatatatgcaactgtctagcctcacatctgtcgactctgccgtctacttttgcgagcgattctactatggcaacacttttgccatggactactgggggcaggggacatcagtaacagttagttctggagggggcggttccgggggcgggggatccggagggggaggcagtgatgtgctgatgacccagataccgttgtcactcccggtctcactgggtgaccaggcaagcatcagctgcaggagcagccagtccatcgtgcactctaacggaaatacctacctggagtggtatctgcagaaacctggccagtcccctaagttgttgatttacaaagtttcaaaccgatttagtggagttcccgataggttttccggttccgggagcggtacagacttcaccctgaagataagtcgggttgaggctgaagacctgggagtatattattgctttcagggcagccacgtaccattcacatttgggagtggaaccaaactggagatcaaaagaaccacaacacctgctccaaggccccccacacccgctccaactatagccagccaaccattgagcctcagacctgaagcttgcaggcccgcagcaggaggcgccgtccatacgcgaggcctggacttcgcgtgtgatatttatatttgggcccctttggccggaacatgtggggtgttgcttctctcccttgtgatcactctgtattgtaagcgcgggagaaagaagctcctgtacatcttcaagcagccttttatgcgacctgtgcaaaccactcaggaagaagatgggtgttcatgccgcttccccgaggaggaagaaggagggtgtgaactgagggtgaaattttctagaagcgccgatgctcccgcatatcagcagggtcagaatcagctctacaatgaattgaatctcggcaggcgagaagagtacgatgttctggacaagagacggggcagggatcccgagatggggggaaagccccggagaaaaaatcctcaggaggggttgtacaatgagctgcagaaggacaagatggctgaagcctatagcgagatcggaatgaaaggcgaaagacgcagaggcaaggggcatgacggtctgtaccagggtctctctacagccaccaaggacacttatgatgcgttgcatatgcaagccttgccaccccgctaa

SEQ ID NO: 32 - DNA, 1479 bp, synthetic construct
  misc_feature 1..1479: note = Made in Lab - anti-CD79A-01_LH CAR polynucleotide construct
  source 1..1479: mol_type = other DNA
atggctctgcctgtgacggccctgcttttgcccctcgccctgcttctgcatgccgcgagacccgacgtgttgatgacccaaataccgcttagtctgcctgtatctcttggggaccaggctagcatctcatgccgcagcagtcaatccattgtgcactcaaatgggaacacctatttggagtggtatctgcaaaaaccgggacagtctccgaaactgctgatatacaaagtaagcaacaggttcagcggagttcctgacagattcagcggaagcggttctggaactgactttacacttaagatctctcgcgttgaggcggaggacctgggcgtgtattactgttttcaaggatcccacgtcccgtttacattcggatcaggcaccaagctggagatcaagcgcggtggcgggggttctggcgggggcggatccggaggcggcggatcccaggtgcagctgcagcagtctggaccagaactggttaagcccggagcttcagttaagatttcctgtaaggcttcaggctatacattttccacttcttggatgaactgggtgaaacagcgccctggccaggggctggaatggatcggacggatctatcccggcgatggagacactaattataacggtaagttcaaagggaaggccaccctcacggccgacaagtcctccaatacagcgtacatgcaactcagttccctgaccagcgttgatagcgcagtttacttctgtgagcgcttctattacggaaacaccttcgctatggattactggggtcaggggacctccgtgaccgtgtcctctaccacaacacctgctccaaggccccccacacccgctccaactatagccagccaaccattgagcctcagacctgaagcttgcaggcccgcagcaggaggcgccgtccatacgcgaggcctggacttcgcgtgtgatatttatatttgggcccctttggccggaacatgtggggtgttgcttctctcccttgtgatcactctgtattgtaagcgcgggagaaagaagctcctgtacatcttcaagcagccttttatgcgacctgtgcaaaccactcaggaagaagatgggtgttcatgccgcttccccgaggaggaagaaggagggtgtgaactgagggtgaaattttctagaagcgccgatgctcccgcatatcagcagggtcagaatcagctctacaatgaattgaatctcggcaggcgagaagagtacgatgttctggacaagagacggggcagggatcccgagatggggggaaagccccggagaaaaaatcctcaggaggggttgtacaatgagctgcagaaggacaagatggctgaagcctatagcgagatcggaatgaaaggcgaaagacgcagaggcaaggggcatgacggtctgtaccagggtctctctacagccaccaaggacacttatgatgcgttgcatatgcaagccttgccaccccgctaa

SEQ ID NO: 33 - DNA, 1482 bp, synthetic construct
  misc_feature 1..1482: note = Made in Lab - anti-CD79A-10_HL CAR polynucleotide construct
  source 1..1482: mol_type = other DNA
atggctctgccagtgactgcgctgctgctgcccctcgctcttctgctgcacgccgctcggccacaggtccaactgcaacagagcggccccgagctggtaaaacccggggcctccgtaaaaatatcctgcaagaccagcggctatgccttttcattctcctggatgaactgggtgaagtggggacccggtcagggacttgagtggatcgggcgaatctatcccggaaacggggacacgaattacaacggcaaatttaaaggcaaggctactctgactgctgacaaaagtagcaacaccgcctacatgcagttgtcctctttgacatcagtagactctgcagtgtatttttgcgcccggtgggtttactccggaaataactacgcggttgactattggggacagggcacctccgtgacagtgtcttctggcggcgggggatcaggtggcggcgggtctgggggtggagggagcgacgtggttatgacccagacccctttgagcctgcccgtgagccttggcgaccaagcctccatctcttgccggtcctctcaatcactggtgcacagtaacgggaatacttatctccactggtatttgcaaaagcccggtcagtctcctaagcttctgatctataaggtgtccaaccgcttttctggagtgcccgatagattttccggatctggatccggaacagacttcacattgaagattagtagagtcgaagcggaggacttgggtgtttatttttgttcccagagtacccacgtgcctccatacacgtttggaggtggaaccaaacttgaaattaagaccacaacacctgctccaaggccccccacacccgctccaactatagccagccaaccattgagcctcagacctgaagcttgcaggcccgcagcaggaggcgccgtccatacgcgaggcctggacttcgcgtgtgatatttatatttgggcccctttggccggaacatgtggggtgttgcttctctcccttgtgatcactctgtattgtaagcgcgggagaaagaagctcctgtacatcttcaagcagccttttatgcgacctgtgcaaaccactcaggaagaagatgggtgttcatgccgcttccccgaggaggaagaaggagggtgtgaactgagggtgaaattttctagaagcgccgatgctcccgcatatcagcagggtcagaatcagctctacaatgaattgaatctcggcaggcgagaagagtacgatgttctggacaagagacggggcagggatcccgagatggggggaaagccccggagaaaaaatcctcaggaggggttgtacaatgagctgcagaaggacaagatggctgaagcctatagcgagatcggaatgaaaggcgaaagacgcagaggcaaggggcatgacggtctgtaccagggtctctctacagccaccaaggacacttatgatgcgttgcatatgcaagccttgccaccccgctaa

SEQ ID NO: 34 - DNA, 1482 bp, synthetic construct
  misc_feature 1..1482: note = Made in Lab - anti-CD79A-10_LH CAR polynucleotide construct
  source 1..1482: mol_type = other DNA
atggccctgccagtaacagcactgctccttcctctcgcactcctcctgcacgcagcaagaccagatgtcgtgatgactcagacacctcttagcttgcccgtctccttgggtgatcaggctagcatttcatgtagatcaagccagagcttggtacattcaaatggcaatacctacctgcactggtatctccagaaacctggccagagcccaaaattgcttatctataaagttagtaacagattctccggggtcccagatcgattttccggctcaggctcaggcacggattttaccctgaagatctcacgagtcgaggcagaagatcttggcgtgtacttttgttcccagagtacccacgtacccccttacacattcggaggagggaccaagttggagatcaaaggaggggggggcagtggggggggcggttccggagggggaggaagccaagtacaactgcaacaaagcggacccgagctcgtcaaacctggtgctagcgtcaaaatttcctgtaagaccagcggctacgcttttagcttttcttggatgaactgggtgaaatgggggccggggcagggcctggagtggataggacgaatttatcccgggaatggggatacaaattacaatggtaaattcaaggggaaagccacactgactgcagataaaagctccaacacggcatacatgcagctcagctccctcacttctgtggattctgctgtttacttttgtgccaggtgggtttactctggtaataactatgccgtggattactgggggcaaggcacctctgttacagtgagttccaccacaacacctgctccaaggccccccacacccgctccaactatagccagccaaccattgagcctcagacctgaagcttgcaggcccgcagcaggaggcgccgtccatacgcgaggcctggacttcgcgtgtgatatttatatttgggcccctttggccggaacatgtggggtgttgcttctctcccttgtgatcactctgtattgtaagcgcgggagaaagaagctcctgtacatcttcaagcagccttttatgcgacctgtgcaaaccactcaggaagaagatgggtgttcatgccgcttccccgaggaggaagaaggagggtgtgaactgagggtgaaattttctagaagcgccgatgctcccgcatatcagcagggtcagaatcagctctacaatgaattgaatctcggcaggcgagaagagtacgatgttctggacaagagacggggcagggatcccgagatggggggaaagccccggagaaaaaatcctcaggaggggttgtacaatgagctgcagaaggacaagatggctgaagcctatagcgagatcggaatgaaaggcgaaagacgcagaggcaaggggcatgacggtctgtaccagggtctctctacagccaccaaggacacttatgatgcgttgcatatgcaagccttgccaccccgctaa

SEQ ID NO: 35 - DNA, 1458 bp, synthetic construct
  misc_feature 1..1458: note = Made in Lab - anti-CD79A-02_HL CAR polynucleotide construct
  source 1..1458: mol_type = other DNA
atggcgcttcctgtcactgccctgcttctgcccctcgctcttctgctgcacgccgctcgccccgaagttcagctgttggaaagcggaggcggcctggttcaacccggtggcagtctgaggctgtcctgcgccgcctccggtcttacattcacatcttacgctatgaattgggtgcgccaagcccccggcaagggcctggagtgggttagtggtatcagcgggtccggaggagggacttactacgccgactctgtaaagggacggttcactatctcccgggacaactccaaaaacacactttacctgcagatgaactccttgcgagccgaagacacagccgtgtactactgtgctaagcttggaggctggagtgattattggggtcaggggaccttggtgacagtgtcttccgggggtgggggatccggtggcggtggatcaggagggggtggctcccagagcgctctcacacagccggccagtgtgtcaggatcacctggacagtccattacgatctcttgcactggaacaagctctgactttggctcctataatctcgtgtcctggtatcagcagcaccccgggaaggctcccaagcttatgatttacgagggctcaaaacgcccttcaggtgtatccaaccgattcagcggaagcaaatccggcaataccgcaagtctcaccataagtggcctgcaggcagaagacgaagccgactactattgttgttcttatgccggcggctcaacatgggtgttcggcgggggcaccaagctgactgtattgaccacaacacctgctccaaggccccccacacccgctccaactatagccagccaaccattgagcctcagacctgaagcttgcaggcccgcagcaggaggcgccgtccatacgcgaggcctggacttcgcgtgtgatatttatatttgggcccctttggccggaacatgtggggtgttgcttctctcccttgtgatcactctgtattgtaagcgcgggagaaagaagctcctgtacatcttcaagcagccttttatgcgacctgtgcaaaccactcaggaagaagatgggtgttcatgccgcttccccgaggaggaagaaggagggtgtgaactgagggtgaaattttctagaagcgccgatgctcccgcatatcagcagggtcagaatcagctctacaatgaattgaatctcggcaggcgagaagagtacgatgttctggacaagagacggggcagggatcccgagatggggggaaagccccggagaaaaaatcctcaggaggggttgtacaatgagctgcagaaggacaagatggctgaagcctatagcgagatcggaatgaaaggcgaaagacgcagaggcaaggggcatgacggtctgtaccagggtctctctacagccaccaaggacacttatgatgcgttgcatatgcaagccttgccaccccgctaa

SEQ ID NO: 36 - DNA, 1458 bp, synthetic construct
  misc_feature 1..1458: note = Made in Lab - anti-CD79A-02_LH CAR polynucleotide construct
  source 1..1458: mol_type = other DNA
atggctctgcctgtaactgctctgctgcttccccttgctctgctcctgcatgccgcccggccgcaaagcgccctgactcagccagcttccgtgtctggctctccggggcagtccatcaccatctcatgcacaggaacctccagcgacttcggatcatataacctggtttcatggtatcagcagcatcctgggaaggctccgaagttgatgatctacgagggaagcaagaggcccagtggggtcagtaaccgcttctctggaagtaagtcaggcaataccgctagtctgaccatctccggattgcaagctgaggacgaagctgattactactgctgttcatatgcagggggttctacttgggtgttcggcggtggaaccaagcttaccgttctgggaggcggaggctccgggggaggcggatcaggcggaggtggatccgaagtgcagctgcttgagtcaggagggggattggtccagccggggggatcattgaggctgtcttgtgccgcaagtggactcacttttaccagttatgcaatgaactgggtgcggcaggcacccgggaagggactggaatgggtgagtggcatatctggcagcgggggcggaacttactacgctgattctgtcaagggaaggtttactatctcacgagacaacagcaaaaacaccctctacctgcagatgaactcactcagagcagaggatactgcagtctactattgtgctaagctgggtggttggagcgactactggggacaagggacgttggtgaccgtgtcttcaaccacaacacctgctccaaggccccccacacccgctccaactatagccagccaaccattgagcctcagacctgaagcttgcaggcccgcagcaggaggcgccgtccatacgcgaggcctggacttcgcgtgtgatatttatatttgggcccctttggccggaacatgtggggtgttgcttctctcccttgtgatcactctgtattgtaagcgcgggagaaagaagctcctgtacatcttcaagcagccttttatgcgacctgtgcaaaccactcaggaagaagatgggtgttcatgccgcttccccgaggaggaagaaggagggtgtgaactgagggtgaaattttctagaagcgccgatgctcccgcatatcagcagggtcagaatcagctctacaatgaattgaatctcggcaggcgagaagagtacgatgttctggacaagagacggggcagggatcccgagatggggggaaagccccggagaaaaaatcctcaggaggggttgtacaatgagctgcagaaggacaagatggctgaagcctatagcgagatcggaatgaaaggcgaaagacgcagaggcaaggggcatgacggtctgtaccagggtctctctacagccaccaaggacacttatgatgcgttgcatatgcaagccttgccaccccgctaa

SEQ ID NO: 37 - protein, 226 aa, Homo sapiens
MPGGPGVLQALPATIFLLFLLSAVYLGPGCQALWMHKVPASLMVSLGEDAHFQCPHNSSNNANVTWWRVLHGNYTWPPEFLGPGEDPNGTLIIQNVNKSHGGIYVCRVQEGNESYQQSCGTYLRVRQPPPRPFLDMGEGTKNRIITAEGIILLFCAVVPGTLLLFRKRWQNEKLGLDAGDEYEDENLYEGLNLDDCSMYEDISRGLQGTYQDVGSLNIGDVQLEKP

SEQ ID NO: 38 - protein, 188 aa, Homo sapiens
MPGGPGVLQALPATIFLLFLLSAVYLGPGCQALWMHKVPASLMVSLGEDAHFQCPHNSSNNANVTWWRVLHGNYTWPPEFLGPGEDPNEPPPRPFLDMGEGTKNRIITAEGIILLFCAVVPGTLLLFRKRWQNEKLGLDAGDEYEDENLYEGLNLDDCSMYEDISRGLQGTYQDVGSLNIGDVQLEKP

SEQ ID NO: 39 - protein, 5 aa, synthetic construct
  REGION 1..5: note = Exemplary linker sequence
DGGGS

SEQ ID NO: 40 - protein, 5 aa, synthetic construct
  REGION 1..5: note = Exemplary linker sequence
TGEKP

SEQ ID NO: 41 - protein, 4 aa, synthetic construct
  REGION 1..4: note = Exemplary linker sequence
GGRR

SEQ ID NO: 42 - protein, 5 aa, synthetic construct
  REGION 1..5: note = Exemplary linker sequence
GGGGS

SEQ ID NO: 43 - protein, 14 aa, synthetic construct
  REGION 1..14: note = Exemplary linker sequence
EGKSSGSGSESKVD

SEQ ID NO: 44 - protein, 18 aa, synthetic construct
  REGION 1..18: note = Exemplary linker sequence
KESGSVSSEQLAQFRSLD

SEQ ID NO: 45 - protein, 8 aa, synthetic construct
  REGION 1..8: note = Exemplary linker sequence
GGRRGGGS

SEQ ID NO: 46 - protein, 9 aa, synthetic construct
  REGION 1..9: note = Exemplary linker sequence
LRQRDGERP

SEQ ID NO: 47 - protein, 12 aa, synthetic construct
  REGION 1..12: note = Exemplary linker sequence
LRQKDGGGSERP

SEQ ID NO: 48 - protein, 16 aa, synthetic construct
  REGION 1..16: note = Exemplary linker sequence
LRQKDGGGSGGGSERP

SEQ ID NO: 49 - protein, 18 aa, synthetic construct
  REGION 1..18: note = Exemplary linker sequence
GSTSGSGKPGSGEGSTKG

SEQ ID NO: 50 - skipped

SEQ ID NO: 51 - protein, 7 aa, synthetic construct
  REGION 1..7: note = Cleavage sequence by TEV protease
ENLYFQG

SEQ ID NO: 52 - protein, 7 aa, synthetic construct
  REGION 1..7: note = Cleavage sequence by TEV protease
ENLYFQS

SEQ ID NO: 53 - protein, 22 aa, synthetic construct
  REGION 1..22: note = Self-cleaving polypeptide comprising 2A site
GSGATNFSLLKQAGDVEENPGP

SEQ ID NO: 54 - protein, 19 aa, synthetic construct
  REGION 1..19: note = Self-cleaving polypeptide comprising 2A site
ATNFSLLKQAGDVEENPGP

SEQ ID NO: 55 - protein, 14 aa, synthetic construct
  REGION 1..14: note = Self-cleaving polypeptide comprising 2A site
LLKQAGDVEENPGP

SEQ ID NO: 56 - protein, 21 aa, synthetic construct
  REGION 1..21: note = Self-cleaving polypeptide comprising 2A site
GSGEGRGSLLTCGDVEENPGP

SEQ ID NO: 57 - protein, 18 aa, synthetic construct
  REGION 1..18: note = Self-cleaving polypeptide comprising 2A site
EGRGSLLTCGDVEENPGP

SEQ ID NO: 58 - protein, 13 aa, synthetic construct
  REGION 1..13: note = Self-cleaving polypeptide comprising 2A site
LLTCGDVEENPGP

SEQ ID NO: 59 - protein, 23 aa, synthetic construct
  REGION 1..23: note = Self-cleaving polypeptide comprising 2A site
GSGQCTNYALLKLAGDVESNPGP

SEQ ID NO: 60 - protein, 20 aa, synthetic construct
  REGION 1..20: note = Self-cleaving polypeptide comprising 2A site
QCTNYALLKLAGDVESNPGP

SEQ ID NO: 61 - protein, 14 aa, synthetic construct
  REGION 1..14: note = Self-cleaving polypeptide comprising 2A site
LLKLAGDVESNPGP

SEQ ID NO: 62 - protein, 25 aa, synthetic construct
  REGION 1..25: note = Self-cleaving polypeptide comprising 2A site
GSGVKQTLNFDLLKLAGDVESNPGP

SEQ ID NO: 63 - protein, 22 aa, synthetic construct
  REGION 1..22: note = Self-cleaving polypeptide comprising 2A site
VKQTLNFDLLKLAGDVESNPGP

SEQ ID NO: 64 - protein, 14 aa, synthetic construct
  REGION 1..14: note = Self-cleaving polypeptide comprising 2A site
LLKLAGDVESNPGP

SEQ ID NO: 65 - protein, 19 aa, synthetic construct
  REGION 1..19: note = Self-cleaving polypeptide comprising 2A site
LLNFDLLKLAGDVESNPGP

SEQ ID NO: 66 - protein, 19 aa, synthetic construct
  REGION 1..19: note = Self-cleaving polypeptide comprising 2A site
TLNFDLLKLAGDVESNPGP

SEQ ID NO: 67 - protein, 14 aa, synthetic construct
  REGION 1..14: note = Self-cleaving polypeptide comprising 2A site
LLKLAGDVESNPGP

SEQ ID NO: 68 - protein, 17 aa, synthetic construct
  REGION 1..17: note = Self-cleaving polypeptide comprising 2A site
NFDLLKLAGDVESNPGP

SEQ ID NO: 69 - protein, 20 aa, synthetic construct
  REGION 1..20: note = Self-cleaving polypeptide comprising 2A site
QLLNFDLLKLAGDVESNPGP

SEQ ID NO: 70 - protein, 24 aa, synthetic construct
  REGION 1..24: note = Self-cleaving polypeptide comprising 2A site
APVKQTLNFDLLKLAGDVESNPGP

SEQ ID NO: 71 - protein, 40 aa, synthetic construct
  REGION 1..40: note = Self-cleaving polypeptide comprising 2A site
VTELLYRMKRAETYCPRPLLAIHPTEARHKQKIVAPVKQT

SEQ ID NO: 72 - protein, 18 aa, synthetic construct
  REGION 1..18: note = Self-cleaving polypeptide comprising 2A site
LNFDLLKLAGDVESNPGP

SEQ ID NO: 73 - protein, 40 aa, synthetic construct
  REGION 1..40: note = Self-cleaving polypeptide comprising 2A site
LLAIHPTEARHKQKIVAPVKQTLNFDLLKLAGDVESNPGP

SEQ ID NO: 74 - protein, 33 aa, synthetic construct
  REGION 1..33: note = Self-cleaving polypeptide comprising 2A site
EARHKQKIVAPVKQTLNFDLLKLAGDVESNPGP

SEQ ID NO: 75 - DNA, 10 bp, synthetic construct
  misc_feature 1..10: note = Consensus Kozak sequence
  source 1..10: mol_type = other DNA
gccrccatgg

SEQ ID NO: 76-77 - skipped (2 entries)

SEQ ID NO: 78 - protein, 5 aa, synthetic construct
  REGION 1..5: note = Exemplary rule for determining heavy chain CDR-H2motif
LEWIG

SEQ ID NO: 79 - skipped